European Patent Specification EP 3 480 310 B1, published November 26, 2025. Title: probe for nucleic acid enrichment and capture and  design method thereof. Applicant: Xiamen Amoy Diagnostics Co.,LTD. The sequence listing filed with the application follows.

SEQUENCE LISTING (51 sequences)

SEQ ID NO: 1 - DNA, 59 bp, Artificial Sequence
  Synthesized
tggttcacccagccttccctggctccctccccatttcctctcatgggcatttcttctaa

SEQ ID NO: 2 - DNA, 59 bp, Artificial Sequence
  Synthesized
ggctccctccccatttcctctcatgggcatttcttctaataaaatctgcagaccatatt

SEQ ID NO: 3 - DNA, 59 bp, Artificial Sequence
  Synthesized
tcatgggcatttcttctaataaaatctgcagaccatattgggtctaatcccatctccag

SEQ ID NO: 4 - DNA, 59 bp, Artificial Sequence
  Synthesized
aaaatctgcagaccatattgggtctaatcccatctccagtctgcttcttggaggaacca

SEQ ID NO: 5 - DNA, 59 bp, Artificial Sequence
  Synthesized
ggtctaatcccatctccagtctgcttcttggaggaaccagactaacatgactctgccct

SEQ ID NO: 6 - DNA, 59 bp, Artificial Sequence; identical to SEQ ID NO: 1
  Synthesized

SEQ ID NO: 7 - DNA, 59 bp, Artificial Sequence
  Synthesized
gattagacccaatatggtctgcagattttattagaagaaatgcccatgagaggaaatgg

SEQ ID NO: 8 - DNA, 59 bp, Artificial Sequence; identical to SEQ ID NO: 4
  Synthesized

SEQ ID NO: 9 - DNA, 59 bp, Artificial Sequence
  Synthesized
tgtattatatagggcagagtcatgttagtctggttcctccaagaagcagactggagatg

SEQ ID NO: 10 - DNA, 59 bp, Artificial Sequence
  Synthesized
actaacatgactctgccctatataatacaaataattattttccatatatctgattttta

SEQ ID NO: 11 - DNA, 35 bp, Artificial Sequence
  Synthesized
ggccgccctggtcctggctttctccggcatcatga

SEQ ID NO: 12 - DNA, 35 bp, Artificial Sequence
  Synthesized
ttggtgagtgcacagagccccagggactcccaagg

SEQ ID NO: 13 - DNA, 40 bp, Artificial Sequence
  Synthesized
gggcaggaaggcaggactgaatagtgtctcaggctgtgcc

SEQ ID NO: 14 - DNA, 48 bp, Artificial Sequence
  Synthesized
acaggtgccaaggtgtcacttcgttatgctagtccctggaattgggtg

SEQ ID NO: 15 - DNA, 35 bp, Artificial Sequence
  Synthesized
gggtggtgattagggcagcccaggccaagccaaaa

SEQ ID NO: 16 - DNA, 35 bp, Artificial Sequence; identical to SEQ ID NO: 11
  Synthesized

SEQ ID NO: 17 - DNA, 36 bp, Artificial Sequence
  Synthesized
gctctgtgcactcaccaatcatgatgccggagaaag

SEQ ID NO: 18 - DNA, 35 bp, Artificial Sequence; identical to SEQ ID NO: 12
  Synthesized

SEQ ID NO: 19 - DNA, 35 bp, Artificial Sequence
  Synthesized
agtcctgccttcctgcccccttgggagtccctggg

SEQ ID NO: 20 - DNA, 40 bp, Artificial Sequence; identical to SEQ ID NO: 13
  Synthesized

SEQ ID NO: 21 - DNA, 59 bp, Artificial Sequence
  Synthesized
tccttctctctctgtcatagggactctggatcccagaaggtgagaaagttaaaattccc

SEQ ID NO: 22 - DNA, 59 bp, Artificial Sequence
  Synthesized
ggactctggatcccagaaggtgagaaagttaaaattcccgtcgctatcaaggaattaag

SEQ ID NO: 23 - DNA, 59 bp, Artificial Sequence
  Synthesized
tgagaaagttaaaattcccgtcgctatcaaggaattaagagaagcaacatctccgaaag

SEQ ID NO: 24 - DNA, 59 bp, Artificial Sequence
  Synthesized
tcgctatcaaggaattaagagaagcaacatctccgaaagccaacaaggaaatcctcgat

SEQ ID NO: 25 - DNA, 59 bp, Artificial Sequence
  Synthesized
gaagcaacatctccgaaagccaacaaggaaatcctcgatgtgagtttctgctttgctgt

SEQ ID NO: 26 - DNA, 59 bp, Artificial Sequence; identical to SEQ ID NO: 21
  Synthesized

SEQ ID NO: 27 - DNA, 59 bp, Artificial Sequence
  Synthesized
atgttgcttctcttaattccttgatagcgacgggaattttaactttctcaccttctggg

SEQ ID NO: 28 - DNA, 59 bp, Artificial Sequence; identical to SEQ ID NO: 24
  Synthesized

SEQ ID NO: 29 - DNA, 59 bp, Artificial Sequence
  Synthesized
tggacccccacacagcaaagcagaaactcacatcgaggatttccttgttggctttcgga

SEQ ID NO: 30 - DNA, 59 bp, Artificial Sequence
  Synthesized
caagtactttgcaaacacacataccttatctcaaggatatagtatgtaattctacatcc

SEQ ID NO: 31 - DNA, 59 bp, Artificial Sequence
  Synthesized
ataccttatctcaaggatatagtatgtaattctacatccattatcttcagctttctccc

SEQ ID NO: 32 - DNA, 59 bp, Artificial Sequence
  Synthesized
agtatgtaattctacatccattatcttcagctttctcccactgtattgaatttttactc

SEQ ID NO: 33 - DNA, 59 bp, Artificial Sequence
  Synthesized
ttatcttcagctttctcccactgtattgaatttttactcccttctagtaatttgggaat

SEQ ID NO: 34 - DNA, 59 bp, Artificial Sequence
  Synthesized
ctgtattgaatttttactcccttctagtaatttgggaatgcctggtttatttgggactc

SEQ ID NO: 35 - DNA, 59 bp, Artificial Sequence; identical to SEQ ID NO: 30
  Synthesized

SEQ ID NO: 36 - DNA, 59 bp, Artificial Sequence
  Synthesized
ttcaatacagtgggagaaagctgaagataatggatgtagaattacatactatatccttg

SEQ ID NO: 37 - DNA, 59 bp, Artificial Sequence; identical to SEQ ID NO: 33
  Synthesized

SEQ ID NO: 38 - DNA, 59 bp, Artificial Sequence
  Synthesized
ccctaaagctggagtcccaaataaaccaggcattcccaaattactagaagggagtaaaa

SEQ ID NO: 39 - DNA, 59 bp, Artificial Sequence
  Synthesized
cctggtttatttgggactccagctttagggaaaaaaagaaaatattggttgatatgttt

SEQ ID NO: 40 - DNA, 59 bp, Artificial Sequence
  Synthesized
gggaaaacacccttcgggatattatccaggagaacttccccaacctagcaagacaggcc

SEQ ID NO: 41 - DNA, 59 bp, Artificial Sequence
  Synthesized
gtgttctctgtgtttgccgaatttgcatgttggcctgtcttgctaggttggggaagttc

SEQ ID NO: 42 - DNA, 59 bp, Artificial Sequence
  Synthesized
acatgcaaattcggcaaacacagagaacaccattaagatactccacgagaagatcaacc

SEQ ID NO: 43 - DNA, 59 bp, Artificial Sequence
  Synthesized
ccttggagaatctgatgattatgtgtcttggggttgatcttctcgtggagtatcttaat

SEQ ID NO: 44 - DNA, 59 bp, Artificial Sequence
  Synthesized
caagacacataatcatcagattctccaaggttgaaatcaagtaaaaactgttaagggca

SEQ ID NO: 45 - DNA, 59 bp, Artificial Sequence
  Synthesized
agaaatgcagcatccatttctatagctccaggctgtgcttttcccctgcgggagccagc

SEQ ID NO: 46 - DNA, 59 bp, Artificial Sequence
  Synthesized
gacaagtcttgggaccaagctgtccagcctcgctggctcccgcaggggaaaagcacagc

SEQ ID NO: 47 - DNA, 59 bp, Artificial Sequence
  Synthesized
aggctggacagcttggtcccaagacttgtcgccacaacccaacacaccagctgtggtag

SEQ ID NO: 48 - DNA, 59 bp, Artificial Sequence
  Synthesized
gttagacctgaagaggcactctggccgctgactaccacagctggtgtgttgggttgtgg

SEQ ID NO: 49 - DNA, 59 bp, Artificial Sequence
  Synthesized
cagcggccagagtgcctcttcaggtctaaccctcacccatccttcctcagtgggtgggg

SEQ ID NO: 50 - DNA, 30 bp, Artificial Sequence
  Synthesized
tgagaaagttaaaattcccgtcgctatcaa

SEQ ID NO: 51 - DNA, 30 bp, Artificial Sequence
  Synthesized
cgaaagccaacaaggaaatcctcgatgtga